European Patent Specification EP 3 483 176 B1, published August 21, 2024. Title: MUTATED IMMUNOGLOBULIN-BINDING PROTEIN HAVING INCREASED ALKALINE TOLERANCE. Applicant: AMICOGEN, INC. The sequence listing filed with the application follows.

SEQUENCE LISTING (32 sequences)

SEQ ID NO: 1 - DNA, 174 bp, Staphylococcus aureus
  polyneclotide sequence of protein A domain A
gctgacaacaatttcaacaaagaacaacaaaatgctttctatgaaatcttgaacatgcctaacttgaacgaagaacaacgcaatggtttcatccaaagcttaaaggatgacccaagtcaaagtgctaaccttttagcagaagctaaaaagttaaatgaatctcaagcaccgaaa

SEQ ID NO: 2 - protein, 58 aa, Staphylococcus aureus.
  amino acid sequence of protein A domain A
ADNNFNKEQQNAFYEILNMPNLNEEQRNGFIQSLKDDPSQSANLLAEAKKLNESQAPK

SEQ ID NO: 3 - protein, 58 aa, Artificial Sequence
  mutant of protein A domain A(AEP1, N18H)
ADNNFNKEQQNAFYEILHMPNLNEEQRNGFIQSLKDDPSQSANLLAEAKKLNESQAPK

SEQ ID NO: 4 - protein, 58 aa, Artificial Sequence
  mutant of protein A domain A(AEP4, D36V)
ADNNFNKEQQNAFYEILNMPNLNEEQRNGFIQSLKVDPSQSANLLAEAKKLNESQAPK

SEQ ID NO: 5 - protein, 58 aa, Artificial Sequence
  mutant of protein A domain A(AEP5, N43Y/L)
ADNNFNKEQQNAFYEILNMPNLNEEQRNGFIQSLKDDPSQSAYLLAEAKKLNESQAPK

SEQ ID NO: 6 - protein, 58 aa, Artificial Sequence
  mutant of protein A domain A(AEP6, N53S)
ADNNFNKEQQNAFYEILNMPNLNEEQRNGFIQSLKDDPSQSANLLAEAKKLSESQAPK

SEQ ID NO: 7 - protein, 58 aa, Artificial Sequence
  mutant of protein A domain A(AEP2, N23L)
ADNNFNKEQQNAFYEILNMPNLTEEQRNGFIQSLKDDPSQSANLLAEAKKLNESQAPK

SEQ ID NO: 8 - protein, 58 aa, Artificial Sequence
  mutant of protein A domain A(AES3, N28W)
ADNNFNKEQQNAFYEILNMPNLNEEQRWGFIQSLKDDPSQSANLLAEAKKLNESQAPK

SEQ ID NO: 9 - protein, 58 aa, Artificial Sequence
  mutant of protein A domain A(maF)
ADNNFNKEQQNAFYEILHMPNLLEEQRWGFIQSLKVDPSQSAYLLAEAKKLSESQAPK

SEQ ID NO: 10 - DNA, 198 bp, Artificial Sequence
  pBC-mAF plasmid
atggctgacaacaatttcaacaaagaacaacaaaatgctttctatgaaatcttgcacatgcctaacttgcttgaagaacaacgctggggtttcatccaaagcttaaaggttgacccaagtcaaagtgcttaccttttagcagaagctaaaaagttaagtgaatctcaagcaccgaaacatcaacatcagcaccaataa

SEQ ID NO: 11 - protein, 239 aa, Artificial Sequence
  amino acid sequence of 4mAF
MADNNFNKEQQNAFYEILHMPNLLEEQRWGFIQSLKVDPSQSAYLLAEAKKLSESQAPKGTADNNFNKEQQNAFYEILHMPNLLEEQRWGFIQSLKVDPSQSAYLLAEAKKLSESQAPKGTADNNFNKEQQNAFYEILHMPNLLEEQRWGFIQSLKVDPSQSAYLLAEAKKLSESQAPKGTADNNFNKEQQNAFYEILHMPNLLEEQRWGFIQSLKVDPSQSAYLLAEAKKLSESQAPK

SEQ ID NO: 12 - DNA, 711 bp, Artificial Sequence
  pET-Fc plasmid
atggacaaaactcacacatgcccaccgtgcccagcacctgaactcctggggggaccgtcagtcttcctcttccccccaaaacccaaggacaccctcatgatctcccggacccctgaggtcacatgcgtggtggtggacgtgagccacgaagaccctgaggtcaagttcaactggtacgtggacggcgtggaggtgcataatgccaagacaaagccgcgggaggagcagtacaacagcacgtaccgtgtggtcagcgtcctcaccgtcctgcaccaggactggctgaatggcaaggagtacaagtgcaaggtctccaacaaagccctcccagcccccatcgagaaaaccatctccaaagccaaagggcagccccgagaaccacaggtgtacaccctgcccccatcccgggaggagatgaccaagaaccaggtcagcctgacctgcctggtcaaaggcttctatcccagcgacatcgccgtggagtgggagagcaatgggcagccggagaacaactacaagaccacgcctcccgtgctggactccgacggctccttcttcctctacagcaagctcaccgtggacaagagcaggtggcagcaggggaacgtcttctcatgctccgtgatgcacgaggctctgcacaaccactacacgcagaagagcctctccctgtctccgggtaaactcgagcaccaccaccaccaccactga

SEQ ID NO: 13 - protein, 236 aa, Artificial Sequence
  amino acid sequence of wild type Fc
MDKTHTCPPCPAPELLGGPSVFLFPPKPKDTLMISRTPEVTCVVVDVSHEDPEVKFNWYVDGVEVHNAKTKPREEQYNSTYRVVSVLTVLHQDWLNGKEYKCKVSNKALPAPIEKTISKAKGQPREPQVYTLPPSREEMTKNQVSLTCLVKGFYPSDIAVEWESNGQPENNYKTTPPVLDSDGSFFLYSKLTVDKSRWQQGNVFSCSVMHEALHNHYTQKSLSLSPGKLEHHHHHH

SEQ ID NO: 14 - DNA, 20 bp, Artificial Sequence
  EP-F primer
gcttgatatcgaattcctgc

SEQ ID NO: 15 - DNA, 20 bp, Artificial Sequence
  T7 primer
taatacgactcactataggg

SEQ ID NO: 16 - DNA, 46 bp, Artificial Sequence
  18-F primer
caaaatgctttctatgaaatcttgnnkatgcctaacttgaacgaag

SEQ ID NO: 17 - DNA, 46 bp, Artificial Sequence
  18-R primer
cttcgttcaagttaggcatmnncaagatttcatagaaagcattttg

SEQ ID NO: 18 - DNA, 43 bp, Artificial Sequence
  23-F primer
cttgaacatgcctaacttgnnkgaagaacaacgcaatggtttc

SEQ ID NO: 19 - DNA, 43 bp, Artificial Sequence
  23-R primer
gaaaccattgcgttgttcttcmnncaagttaggcatgttcaag

SEQ ID NO: 20 - DNA, 40 bp, Artificial Sequence
  28-F primer
gaacgaagaacaacgcnnkggtttcatccaaagcttaaag

SEQ ID NO: 21 - DNA, 40 bp, Artificial Sequence
  28-R primer
ctttaagctttggatgaaaccmnngcgttgttcttcgttc

SEQ ID NO: 22 - DNA, 45 bp, Artificial Sequence
  36-F primer
ggtttcatccaaagcttaaagnnkgacccaagtcaaagtgctaac

SEQ ID NO: 23 - DNA, 45 bp, Artificial Sequence
  36-R primer
gttagcactttgacttgggtcmnnctttaagctttggatgaaacc

SEQ ID NO: 24 - DNA, 44 bp, Artificial Sequence
  43-F primer
atgacccaagtcaaagtgctnnkcttttagcagaagctaaaaag

SEQ ID NO: 25 - DNA, 44 bp, Artificial Sequence
  43-R primer
ctttttagcttctgctaaaagmnnagcactttgacttgggtcat

SEQ ID NO: 26 - DNA, 48 bp, Artificial Sequence
  52-F primer
cttttagcagaagctaaaaagttannkgaatctcaagcaccgaaacat

SEQ ID NO: 27 - DNA, 48 bp, Artificial Sequence
  52-R primer
atgtttcggtgcttgagattcmnntaactttttagcttctgctaaaag

SEQ ID NO: 28 - DNA, 31 bp, Artificial Sequence
  mAF-F primer
cggggtaccgctgacaacaatttcaacaaag

SEQ ID NO: 29 - DNA, 34 bp, Artificial Sequence
  mAF-R primer
cggggtacctttcggtgcttgagattcatttaac

SEQ ID NO: 30 - DNA, 31 bp, Artificial Sequence
  4mAF-F primer
cgccatatggctgacaacaatttcaacaaag

SEQ ID NO: 31 - DNA, 34 bp, Artificial Sequence
  4mAF-R primer
ccgctcgagtttcggtgcttgagattcatttaac

SEQ ID NO: 32 - DNA, 717 bp, Artificial Sequence
  polynuclotide sequence of 4mAF
atggctgacaacaatttcaacaaagaacaacaaaatgctttctatgaaatcttgcacatgcctaacttgcttgaagaacaacgctggggtttcatccaaagcttaaaggttgacccaagtcaaagtgcttaccttttagcagaagctaaaaagttaagtgaatctcaagcaccgaaaggtaccgctgacaacaatttcaacaaagaacaacaaaatgctttctatgaaatcttgcacatgcctaacttgcttgaagaacaacgctggggtttcatccaaagcttaaaggttgacccaagtcaaagtgcttaccttttagcagaagctaaaaagttaagtgaatctcaagcaccgaaaggtaccgctgacaacaatttcaacaaagaacaacaaaatgctttctatgaaatcttgcacatgcctaacttgcttgaagaacaacgctggggtttcatccaaagcttaaaggttgacccaagtcaaagtgcttaccttttagcagaagctaaaaagttaagtgaatctcaagcaccgaaaggtaccgctgacaacaatttcaacaaagaacaacaaaatgctttctatgaaatcttgcacatgcctaacttgcttgaagaacaacgctggggtttcatccaaagcttaaaggttgacccaagtcaaagtgcttaccttttagcagaagctaaaaagttaagtgaatctcaagcaccgaaa